European Patent Specification EP 3 882 275 B1, published September 18, 2024. Title: ANTI-PD-1/VEGFA BIFUNCTIONAL ANTIBODY, PHARMACEUTICAL COMPOSITION THEREOF AND USE THEREOF. Applicant: AKESO BIOPHARMA, INC. The sequence listing filed with the application follows.

SEQUENCE LISTING (26 sequences)

SEQ ID NO: 1 - protein, 171 aa, Artificial
  The amino acid sequence of VEGFA-His
APMAEGGGQNHHEVVKFMDVYQRSYCHPIETLVDIFQEYPDEIEYIFKPSCVPLMRCGGCCNDEGLECVPTEESNITMQIMRIKPHQGQHIGEMSFLQHNKCECRPKKDRARQENPCGPCSERRKHLFVQDPQTCKCSCKNTDSRCKARQLELNERTCRCDKPRRHHHHHH

SEQ ID NO: 2 - DNA, 513 bp, Artificial
  Nucleotide sequence of VEGFA-His
gcacccatggccgagggcggcggccagaaccaccacgaggtggtgaagttcatggacgtgtaccagagaagctactgccaccccatcgagaccctggtggacatcttccaggagtaccccgacgagatcgagtacatcttcaagcccagctgcgtgcccctgatgagatgcggcggctgctgcaacgacgagggcctggagtgcgtgcccaccgaggagagcaacatcaccatgcagatcatgagaatcaagccccaccagggccagcacatcggcgagatgagcttcctgcagcacaacaagtgcgagtgcagacccaagaaggacagagccagacaggagaacccctgcggcccctgcagcgagagaagaaagcacctgttcgtgcaggacccccagacctgcaagtgcagctgcaagaacaccgacagcagatgcaaggccagacagctggagctgaacgagagaacctgcagatgcgacaagcccagaagacatcatcaccatcaccac

SEQ ID NO: 3 - protein, 998 aa, Artificial
  The amino acid sequence of Fusion protein VEGFR2- hFc
MQSKVLLAVALWLCVETRAASVGLPSVSLDLPRLSIQKDILTIKANTTLQITCRGQRDLDWLWPNNQSGSEQRVEVTECSDGLFCKTLTIPKVIGNDTGAYKCFYRETDLASVIYVYVQDYRSPFIASVSDQHGVVYITENKNKTVVIPCLGSISNLNVSLCARYPEKRFVPDGNRISWDSKKGFTIPSYMISYAGMVFCEAKINDESYQSIMYIVVVVGYRIYDVVLSPSHGIELSVGEKLVLNCTARTELNVGIDFNWEYPSSKHQHKKLVNRDLKTQSGSEMKKFLSTLTIDGVTRSDQGLYTCAASSGLMTKKNSTFVRVHEKPFVAFGSGMESLVEATVGERVRIPAKYLGYPPPEIKWYKNGIPLESNHTIKAGHVLTIMEVSERDTGNYTVILTNPISKEKQSHVVSLVVYVPPQIGEKSLISPVDSYQYGTTQTLTCTVYAIPPPHHIHWYWQLEEECANEPSQAVSVTNPYPCEEWRSVEDFQGGNKIEVNKNQFALIEGKNKTVSTLVIQAANVSALYKCEAVNKVGRGERVISFHVTRGPEITLQPDMQPTEQESVSLWCTADRSTFENLTWYKLGPQPLPIHVGELPTPVCKNLDTLWKLNATMFSNSTNDILIMELKNASLQDQGDYVCLAQDRKTKKRHCVVRQLTVLERVAPTITGNLENQTTSIGESIEVSCTASGNPPPQIMWFKDNETLVEDSGIVLKDGNRNLTIRRVRKEDEGLYTCQACSVLGCAKVEAFFIIEGAQEKTNLESRENLYFQGTHTCPPCPAPELLGGPSVFLFPPKPKDTLMISRTPEVTCVVVDVSHEDPEVKFNWYVDGVEVHNAKTKPREEQYNSTYRVVSVLTVLHQDWLNGKEYKCKVSNKALPAPIEKTISKAKGQPREPQVYTLPPSRDELTKNQVSLTCLVKGFYPSDIAVEWESNGQPENNYKTTPPVLDSDGSFFLYSKLTVDKSRWQQGNVFSCSVMHEALHNHYTQKSLSLSPGK

SEQ ID NO: 4 - DNA, 2997 bp, Artificial
  Nucleotide sequence of Fusion protein VEGFR2- hFc
atgcagagcaaggtgctgctggccgtcgccctgtggctctgcgtggagacccgggccgcctctgtgggtttgcctagtgtttctcttgatctgcccaggctcagcatacaaaaagacatacttacaattaaggctaatacaactcttcaaattacttgcaggggacagagggacttggactggctttggcccaataatcagagtggcagtgagcaaagggtggaggtgactgagtgcagcgatggcctcttctgtaagacactcacaattccaaaagtgatcggaaatgacactggagcctacaagtgcttctaccgggaaactgacttggcctcggtcatttatgtctatgttcaagattacagatctccatttattgcttctgttagtgaccaacatggagtcgtgtacattactgagaacaaaaacaaaactgtggtgattccatgtctcgggtccatttcaaatctcaacgtgtcactttgtgcaagatacccagaaaagagatttgttcctgatggtaacagaatttcctgggacagcaagaagggctttactattcccagctacatgatcagctatgctggcatggtcttctgtgaagcaaaaattaatgatgaaagttaccagtctattatgtacatagttgtcgttgtagggtataggatttatgatgtggttctgagtccgtctcatggaattgaactatctgttggagaaaagcttgtcttaaattgtacagcaagaactgaactaaatgtggggattgacttcaactgggaatacccttcttcgaagcatcagcataagaaacttgtaaaccgagacctaaaaacccagtctgggagtgagatgaagaaatttttgagcaccttaactatagatggtgtaacccggagtgaccaaggattgtacacctgtgcagcatccagtgggctgatgaccaagaagaacagcacatttgtcagggtccatgaaaaaccttttgttgcttttggaagtggcatggaatctctggtggaagccacggtgggggagcgtgtcagaatccctgcgaagtaccttggttacccacccccagaaataaaatggtataaaaatggaataccccttgagtccaatcacacaattaaagcggggcatgtactgacgattatggaagtgagtgaaagagacacaggaaattacactgtcatccttaccaatcccatttcaaaggagaagcagagccatgtggtctctctggttgtgtatgtcccaccccagattggtgagaaatctctaatctctcctgtggattcctaccagtacggcaccactcaaacgctgacatgtacggtctatgccattcctcccccgcatcacatccactggtattggcagttggaggaagagtgcgccaacgagcccagccaagctgtctcagtgacaaacccatacccttgtgaagaatggagaagtgtggaggacttccagggaggaaataaaattgaagttaataaaaatcaatttgctctaattgaaggaaaaaacaaaactgtaagtacccttgttatccaagcggcaaatgtgtcagctttgtacaaatgtgaagcggtcaacaaagtcgggagaggagagagggtgatctccttccacgtgaccaggggtcctgaaattactttgcaacctgacatgcagcccactgagcaggagagcgtgtctttgtggtgcactgcagacagatctacgtttgagaacctcacatggtacaagcttggcccacagcctctgccaatccatgtgggagagttgcccacacctgtttgcaagaacttggatactctttggaaattgaatgccaccatgttctctaatagcacaaatgacattttgatcatggagcttaagaatgcatccttgcaggaccaaggagactatgtctgccttgctcaagacaggaagaccaagaaaagacattgcgtggtcaggcagctcacagtcctagagcgtgtggcacccacgatcacaggaaacctggagaatcagacgacaagtattggggaaagcatcgaagtctcatgcacggcatctgggaatccccctccacagatcatgtggtttaaagataatgagacccttgtagaagactcaggcattgtattgaaggatgggaaccggaacctcactatccgcagagtgaggaaggaggacgaaggcctctacacctgccaggcatgcagtgttcttggctgtgcaaaagtggaggcatttttcataatagaaggtgcccaggaaaagacgaacttggaatctagagaaaacctgtattttcagggcactcacacatgcccaccgtgcccagcacctgaactcctggggggaccgtcagtcttcctcttccccccaaaacccaaggacaccctcatgatctcccggacccctgaggtcacatgcgtggtggtggacgtgagccacgaagaccctgaggtcaagttcaactggtacgtggacggcgtggaggtgcataatgccaagacaaagccgcgggaggagcagtacaacagcacgtaccgtgtggtcagcgtcctcaccgtcctgcaccaggactggctgaatggcaaggagtacaagtgcaaggtctccaacaaagccctcccagcccccatcgagaaaaccatctccaaagccaaagggcagccccgagaaccacaggtgtacaccctgcccccatcccgggatgagctgaccaagaaccaggtcagcctgacctgcctggtcaaaggcttctatcccagcgacatcgccgtggagtgggagagcaatgggcagccggagaacaactacaagaccacgcctcccgtgttggactccgacggctccttcttcctctacagcaagctcaccgtggacaagagcaggtggcagcaggggaacgtcttctcatgctccgtgatgcatgaggctctgcacaaccactacacgcagaagagcctctccctgtctcccgggaaatga

SEQ ID NO: 5 - protein, 123 aa, Artificial [sequence omitted]

SEQ ID NO: 6 - DNA, 369 bp, Artificial
  Nucleotide sequence of Bevacizumab heavy chain variable region
gaggtgcagctggtcgagtccgggggggggctggtgcagccaggcgggtctctgaggctgagttgcgccgcttcagggtacaccttcacaaactatggaatgaattgggtgcgccaggcaccaggaaagggactggagtgggtcggctggatcaacacttacaccggggaacctacctatgcagccgactttaagcggcggttcaccttcagcctggatacaagcaaatccactgcctacctgcagatgaacagcctgcgagctgaggacaccgcagtctactattgtgctaaatatccccactactatgggagcagccattggtattttgacgtgtgggggcaggggactctggtgacagtgagcagc

SEQ ID NO: 7 - protein, 107 aa, Artificial [sequence omitted]

SEQ ID NO: 8 - DNA, 321 bp, Artificial
  Nucleotide sequence of Bevacizumab light chain variable region
gatattcagatgactcagagcccctcctccctgtccgcctctgtgggcgacagggtcaccatcacatgcagtgcttcacaggatatttccaactacctgaattggtatcagcagaagccaggaaaagcacccaaggtgctgatctacttcactagctccctgcactcaggagtgccaagccggttcagcggatccggatctggaaccgactttactctgaccatttctagtctgcagcctgaggatttcgctacatactattgccagcagtattctaccgtgccatggacatttggccaggggactaaagtcgagatcaag

SEQ ID NO: 9 - protein, 118 aa, Artificial
  The amino acid sequence of humanized antibody 14C12H1L1 heavy chain variable region
EVQLVESGGGLVQPGGSLRLSCAASGFAFSSYDMSWVRQAPGKGLDWVATISGGGRYTYYPDSVKGRFTISRDNSKNNLYLQMNSLRAEDTALYYCANRYGEAWFAYWGQGTLVTVSS

SEQ ID NO: 10 - DNA, 354 bp, Artificial
  Nucleotide sequence of humanized antibody 14C12H1L1 heavy chain variable region
gaagtgcagctggtcgagtctgggggagggctggtgcagcccggcgggtcactgcgactgagctgcgcagcttccggattcgcctttagctcctacgacatgtcctgggtgcgacaggcaccaggaaagggactggattgggtcgctactatctcaggaggcgggagatacacctactatcctgacagcgtcaagggccggttcacaatctctagagataacagtaagaacaatctgtatctgcagatgaacagcctgagggctgaggacaccgcactgtactattgtgccaaccgctacggggaagcatggtttgcctattgggggcagggaaccctggtgacagtctctagt

SEQ ID NO: 11 - protein, 107 aa, Artificial
  The amino acid sequence of humanized antibody 14C12H1L1 light chain variable region
DIQMTQSPSSMSASVGDRVTFTCRASQDINTYLSWFQQKPGKSPKTLIYRANRLVSGVPSRFSGSGSGQDYTLTISSLQPEDMATYYCLQYDEFPLTFGAGTKLELK

SEQ ID NO: 12 - DNA, 321 bp, Artificial
  Nucleotide sequence of humanized antibody 14C12H1L1 light chain variable region
gacattcagatgactcagagcccctcctccatgtccgcctctgtgggcgacagggtcaccttcacatgccgcgctagtcaggatatcaacacctacctgagctggtttcagcagaagccagggaaaagccccaagacactgatctaccgggctaatagactggtgtctggagtcccaagtcggttcagtggctcagggagcggacaggactacactctgaccatcagctccctgcagcctgaggacatggcaacctactattgcctgcagtatgatgagttcccactgacctttggcgccgggacaaaactggagctgaag

SEQ ID NO: 13 - protein, 20 aa, Artificial
  The amino acid sequence of Linker 1
GGGGSGGGGSGGGGSGGGGS

SEQ ID NO: 14 - protein, 5 aa, Artificial
  linker fragment
GGGGS

SEQ ID NO: 15 - protein, 8 aa, Artificial
  HCDR1 of Antibody Bevacizumab
GYTFTNYG

SEQ ID NO: 16 - protein, 8 aa, Artificial
  HCDR2 of Antibody Bevacizumab
INTYTGEP

SEQ ID NO: 17 - protein, 16 aa, Artificial
  HCDR3 of Antibody Bevacizumab
AKYPHYYGSSHWYFDV

SEQ ID NO: 18 - protein, 6 aa, Artificial
  LCDR1 of Antibody Bevacizumab
QDISNY

SEQ ID NO: 19 - protein, 3 aa, Artificial
  LCDR2 of Antibody Bevacizumab
FTS

SEQ ID NO: 20 - protein, 9 aa, Artificial
  LCDR3 of Antibody Bevacizumab
QQYSTVPWT

SEQ ID NO: 21 - protein, 8 aa, Artificial
  HCDR1 of Antibody 14C12H1L1
GFAFSSYD

SEQ ID NO: 22 - protein, 8 aa, Artificial
  HCDR2 of Antibody 14C12H1L1
ISGGGRYT

SEQ ID NO: 23 - protein, 11 aa, Artificial
  HCDR3 of Antibody 14C12H1L1
ANRYGEAWFAY

SEQ ID NO: 24 - protein, 6 aa, Artificial
  LCDR1 of Antibody 14C12H1L1
QDINTY

SEQ ID NO: 25 - protein, 3 aa, Artificial
  LCDR2 of Antibody 14C12H1L1
RAN

SEQ ID NO: 26 - protein, 9 aa, Artificial
  LCDR3 of Antibody 14C12H1L1
LQYDEFPLT